European Patent Application EP 4 218 938 A1, published August 2, 2023. Title: Treatment of mitochondrial diseases. Applicant: FUNDACIO HOSPITAL UNIVERSITARI VALL D'HEBRON - INSTITUT DE RECERCA. Application EP. The sequence listing filed with the application follows.

SEQUENCE LISTING (13 sequences)

SEQ ID NO: 1 - protein, 1190 aa, Homo sapiens
MSRLLWRKVAGATVGPGPVPAPGRWVSSSVPASDPSDGQRRRQQQQQQQQQQQQQPQQPQVLSSEGGQLRHNPLDIQMLSRGLHEQIFGQGGEMPGEAAVRRSVEHLQKHGLWGQPAVPLPDVELRLPPLYGDNLDQHFRLLAQKQSLPYLEAANLLLQAQLPPKPPAWAWAEGWTRYGPEGEAVPVAIPEERALVFDVEVCLAEGTCPTLAVAISPSAWYSWCSQRLVEERYSWTSQLSPADLIPLEVPTGASSPTQRDWQEQLVVGHNVSFDRAHIREQYLIQGSRMRFLDTMSMHMAISGLSSFQRSLWIAAKQGKHKVQPPTKQGQKSQRKARRGPAISSWDWLDISSVNSLAEVHRLYVGGPPLEKEPRELFVKGTMKDIRENFQDLMQYCAQDVWATHEVFQQQLPLFLERCPHPVTLAGMLEMGVSYLPVNQNWERYLAEAQGTYEELQREMKKSLMDLANDACQLLSGERYKEDPWLWDLEWDLQEFKQKKAKKVKKEPATASKLPIEGAGAPGDPMDQEDLGPCSEEEEFQQDVMARACLQKLKGTTELLPKRPQHLPGHPGWYRKLCPRLDDPAWTPGPSLLSLQMRVTPKLMALTWDGFPLHYSERHGWGYLVPGRRDNLAKLPTGTTLESAGVVCPYRAIESLYRKHCLEQGKQQLMPQEAGLAEEFLLTDNSAIWQTVEELDYLEVEAEAKMENLRAAVPGQPLALTARGGPKDTQPSYHHGNGPYNDVDIPGCWFFKLPHKDGNSCNVGSPFAKDFLPKMEDGTLQAGPGGASGPRALEINKMISFWRNAHKRISSQMVVWLPRSALPRAVIRHPDYDEEGLYGAILPQVVTAGTITRRAVEPTWLTASNARPDRVGSELKAMVQAPPGYTLVGADVDSQELWIAAVLGDAHFAGMHGCTAFGWMTLQGRKSRGTDLHSKTATTVGISREHAKIFNYGRIYGAGQPFAERLLMQFNHRLTQQEAAEKAQQMYAATKGLRWYRLSDEGEWLVRELNLPVDRTEGGWISLQDLRKVQRETARKSQWKKWEVVAERAWKGGTESEMFNKLESIATSDIPRTPVLGCCISRALEPSAVQEEFMTSRVNWVVQSSAVDYLHLMLVAMKWLFEEFAIDGRFCISIHDEVRYLVREEDRYRAALALQITNLLTRCMFAYKLGLNDLPQSVAFFSAVDIDRCLR

SEQ ID NO: 2 - DNA, 19 bp, synthetic construct
  source 1..19: mol_type = other DNA; note = PRIMER
gtccacaccaccaagcagt

SEQ ID NO: 3 - DNA, 20 bp, synthetic construct
  source 1..20: mol_type = other DNA; note = PRIMER
ggtcccaagcactatgctcc

SEQ ID NO: 4 - DNA, 20 bp, synthetic construct
  source 1..20: mol_type = other DNA; note = PRIMER
ccttgctgaatgcaggtgct

SEQ ID NO: 5 - DNA, 22 bp, synthetic construct
  source 1..22: mol_type = other DNA; note = PRIMER
tgtgcctgaaatcacactctgt

SEQ ID NO: 6 - DNA, 20 bp, synthetic construct
  source 1..20: mol_type = other DNA; note = PRIMER
atggtctgctgagtggttgt

SEQ ID NO: 7 - DNA, 21 bp, synthetic construct
  source 1..21: mol_type = other DNA; note = PRIMER
ccctcagagcccagtttctac

SEQ ID NO: 8 - DNA, 20 bp, synthetic construct
  source 1..20: mol_type = other DNA; note = PRIMER
cccagtttatgaccagccgt

SEQ ID NO: 9 - DNA, 20 bp, synthetic construct
  source 1..20: mol_type = other DNA; note = PRIMER
caaggaacgctcacccaaag

SEQ ID NO: 10 - DNA, 20 bp, synthetic construct
  source 1..20: mol_type = other DNA; note = PRIMER
aggggaagccctgctctaag

SEQ ID NO: 11 - DNA, 21 bp, synthetic construct
  source 1..21: mol_type = other DNA; note = PRIMER
acaaatgtgttgtgctcaccc

SEQ ID NO: 12 - DNA, 35 bp, synthetic construct
  source 1..35: mol_type = other DNA; note = PRIMER
accgcccgtcaccctcctcaagtatacttcaaagg

SEQ ID NO: 13 - DNA, 35 bp, synthetic construct
  source 1..35: mol_type = other DNA; note = PRIMER
accgccaggtcctttgagttttaagctgtggctcg